European Patent Application EP 4 717 264 A1, published April 1, 2026. Title: USE OF INTERLEUKIN (IL)-17A INHIBITOR IN PREPARATION OF MEDICAMENT FOR TREATING INFLAMMATORY DISEASE. Applicant: Xiangnan University. The sequence listing filed with the application follows.

SEQUENCE LISTING (10 sequences)

SEQ ID NO: 1 - DNA, 21 bp, synthetic construct
  source 1..21: mol_type = other DNA; note = Forward primer for GAPDH
aggtcggtgtgaacggatttg

SEQ ID NO: 2 - DNA, 23 bp, synthetic construct
  source 1..23: mol_type = other DNA; note = Reverse primer for GAPDH
tgtagaccatgtagttgaggtca

SEQ ID NO: 3 - DNA, 20 bp, synthetic construct
  source 1..20: mol_type = other DNA; note = Forward primer for IL-23
ctcggtgaacaactgaggga

SEQ ID NO: 4 - DNA, 20 bp, synthetic construct
  source 1..20: mol_type = other DNA; note = Rverse primer for IL-23
ggtggaatctctgcccactt

SEQ ID NO: 5 - DNA, 20 bp, synthetic construct
  source 1..20: mol_type = other DNA; note = Forward primer for IL-17A
actacctcaaccgttccacg

SEQ ID NO: 6 - DNA, 19 bp, synthetic construct
  source 1..19: mol_type = other DNA; note = Reverse primer for IL-17A
ttcctccgcattgacacag

SEQ ID NO: 7 - DNA, 21 bp, synthetic construct
  source 1..21: mol_type = other DNA; note = Forward primer for TNF-alpha
atgagcacagaaagcatgatc

SEQ ID NO: 8 - DNA, 22 bp, synthetic construct
  source 1..22: mol_type = other DNA; note = Reverse primer for TNF-alpha
ggtctgggccatagaactgatg

SEQ ID NO: 9 - DNA, 23 bp, synthetic construct
  source 1..23: mol_type = other DNA; note = Forward primer for IL-6
tagtccttcctaccccaatttcc

SEQ ID NO: 10 - DNA, 21 bp, synthetic construct
  source 1..21: mol_type = other DNA; note = Reverse primer for IL-6
ttggtccttagccactccttc